European Patent Application EP 4 129 332 A1, published February 8, 2023. Title: METHOD FOR DISPLAYING BISPECIFIC ANTIBODY ON SURFACE OF MAMMALIAN CELL AND VECTOR. Applicant: DDBio.Co,Ltd.,(Shang Hai). The sequence listing filed with the application follows.

SEQUENCE LISTING (32 sequences)

SEQ ID NO: 1 - DNA, 12 bp, Artificial Sequence
  B2
cgtctcagtggt

SEQ ID NO: 2 - DNA, 12 bp, Artificial Sequence
  B3
cgtctcatcagc

SEQ ID NO: 3 - DNA, 12 bp, Artificial Sequence
  B4
cgtctcaagtcc

SEQ ID NO: 4 - DNA, 12 bp, Artificial Sequence
  B5
cgtctcagctga

SEQ ID NO: 5 - DNA, 12 bp, Artificial Sequence
  B6
cgtctcctctgc

SEQ ID NO: 6 - DNA, 13 bp, Artificial Sequence
  S5
ggccacaggggcc

SEQ ID NO: 7 - DNA, 13 bp, Artificial Sequence
  S6
ggcctgcacggcc

SEQ ID NO: 8 - DNA, 57 bp, Artificial Sequence
  sp1 nucleic acid sequence
atgccctgggctctgctcctcctgaccctcctcactcactctgccgtctcagtggtc

SEQ ID NO: 9 - protein, 19 aa, Artificial Sequence
  sp1 amino acid sequence
MPWALLLLTLLTHSAVSVV

SEQ ID NO: 10 - DNA, 57 bp, Artificial Sequence
  sp2 nucleic acid sequence
atggggtcaaccgccatcctcgccctcctcctggctgttctccaaggcgtctcagct

SEQ ID NO: 11 - protein, 19 aa, Artificial Sequence
  sp2 amino acid sequence
MGSTAILALLLAVLQGVSA

SEQ ID NO: 12 - DNA, 57 bp, Artificial Sequence
  sp3 nucleic acid sequence
atggactggacctggaggatcctcttcttggtggcagcggccacaggggcccactcc

SEQ ID NO: 13 - protein, 19 aa, Artificial Sequence
  sp3 amino acid sequence
MDWTWRILFLVAAATGAHS

SEQ ID NO: 14 - DNA, 37 bp, Artificial Sequence
  P1-I
aaggcctgcacggccctcgagtctagagggcccgttt

SEQ ID NO: 15 - DNA, 86 bp, Artificial Sequence
  P2-I
gggagacccaagctggctagtagtccaccatgccctgggctctgctcctcctgaccctcctcactcactctgccgtctcagtggtc

SEQ ID NO: 16 - DNA, 43 bp, Artificial Sequence
  P3-II
caccgtgaccgtctcatcagctagcaccaagggcccatcggtc

SEQ ID NO: 17 - DNA, 89 bp, Artificial Sequence
  P4-II
tcagctgagacgccttggagaacagccaggaggagggcgaggatggcggttgaccccatggtggttcatagccagcttgggtctcccta

SEQ ID NO: 18 - DNA, 42 bp, Artificial Sequence
  P5-III
accctggtgaccgtctcctctgcctccaccaagggcccatcg

SEQ ID NO: 19 - DNA, 83 bp, Artificial Sequence
  P6-III
tgggcccctgtggccgctgccaccaagaagaggatcctccaggtccagtccatggtggttcatagccagcttgggtctcccta

SEQ ID NO: 20 - DNA, 49 bp, Artificial Sequence
  P7-LC1
tggcagcggccacaggggcccactccgaaattgtgctgacccagagccc

SEQ ID NO: 21 - DNA, 54 bp, Artificial Sequence
  P8-LC1
tagactcgagggccgtgcaggccttatcagcattcgccgcggttaaagcttttg

SEQ ID NO: 22 - DNA, 50 bp, Artificial Sequence
  P9-LC2
actcactctgccgtctcagtggtcgacatccagatgacccagtccccttc

SEQ ID NO: 23 - DNA, 43 bp, Artificial Sequence
  agctgcacctgggacttgagacggcactcgcccctgttgaagc
agctgcacctgggacttgagacggcactcgcccctgttgaagc

SEQ ID NO: 24 - DNA, 44 bp, Artificial Sequence
  P11-VH1
gggcgagtgccgtctcaagtcccaggtgcagctggtgcagagcg

SEQ ID NO: 25 - DNA, 42 bp, Artificial Sequence
  P12-VH1
ccttggtgctagctgatgagacggtcacggtggtgccctggc

SEQ ID NO: 26 - DNA, 44 bp, Artificial Sequence
  P13-VH2
ttctccaaggcgtctcagctgaggtgcagctggtggaaagcggc

SEQ ID NO: 27 - DNA, 42 bp, Artificial Sequence
  P14-VH2
ttggtggaggcagaggagacggtcaccagggtgccctggccc

SEQ ID NO: 28 - DNA, 657 bp, Artificial Sequence
  PD1-LC
gaaattgtgctgacccagagccctgccacactcagcctgagccctggagagagggccaccctgtcctgcagagccagcaagggcgtgagcaccagcggctacagctacctgcactggtaccagcagaagcccggccaggctcccagactgctgatctacctggcttcttatttagaaagcggcgtgcctgctagattcagcggctccggctccggcaccgactttaccctgaccatcagctccctggagcccgaggacttcgccgtgtactactgccagcacagcagggacctgcccctgacctttggcggaggcaccaaggtggagatcaagaggaccgtggccgctcccagcgtgttcatcttcccccccagcgacgagcagctgaagagcggaaccgccagcgtggtgtgcctgctgaacaacttctaccccagggaggccaaggtgcagtggaaggtcgacaacgccctgcagagcggcaatagccaggagtccgtgaccgagcaggacagcaaggacagcacctacagcctgagcagcaccctcaccctgtccaaggccgactacgagaagcataaggtgtacgcctgtgaggtgacccaccagggcctgtccagccctgtgaccaaaagctttaaccgcggcgaatgctga

SEQ ID NO: 29 - DNA, 360 bp, Artificial Sequence
  PD1-VH
caggtgcagctggtgcagagcggcgtggaggtgaaaaagcccggcgccagcgtgaaggtgtcctgtaaggcctccggctacacattcaccaactactacatgtactgggtgaggcaagcccctggccagggactggaatggatgggcggaatcaacccctccaatggaggcaccaactttaacgagaagttcaagaacagggtgacactgacaaccgacagcagcacaacaaccgcttacatggagctgaagagcctgcagttcgatgacaccgccgtgtactactgcgccaggagggactacaggttcgacatgggctttgattactggggccagggcaccaccgtgaccgtctcatca

SEQ ID NO: 30 - DNA, 642 bp, Artificial Sequence
  PDL1-LC
gacatccagatgacccagtccccttccagcctgagcgctagcgtgggcgacagggtgaccatcacctgcagagccagccaggatgtgtctactgctgttgcttggtaccagcagaagcctggcaaggcccccaagctgctgatttactccgccagcttcctgtacagcggcgtgcccagcagatttagcggcagcggctccggcaccgatttcaccctgaccatctccagcctgcagcccgaggacttcgccacctattactgccagcagtacctgtaccaccccgccacctttggccagggcaccaaggtggagatcaagaggaccgtggccgctccttccgtgttcatctttccccccagcgacgagcagctgaagtccggcaccgccagcgtggtgtgtctgctgaacaacttctaccccagggaggccaaggtgcagtggaaggtggacaacgccctgcagtccggcaactcccaggagagcgtgaccgagcaggactccaaggacagcacctacagcctgagcagcaccctgaccctgtccaaggccgactacgagaagcacaaagtgtacgcctgcgaggtgacccaccaaggcctgtccagccccgtgaccaagagcttcaacaggggcgagtgc

SEQ ID NO: 31 - DNA, 354 bp, Artificial Sequence
  PDL1-VH
gaggtgcagctggtggaaagcggcggcggactggtgcagcctggaggctccctcagactgtcctgcgctgcctccggcttcacattcagcgactcctggattcattgggtcagacaggcccctggaaagggcctggagtgggtggcttggatcagcccttacggcggaagcacctactacgccgatagcgtgaagggaaggttcaccatttccgccgacaccagcaagaacaccgcttacctccagatgaacagcctgagggctgaggacacagccgtgtactattgcgccaggagacactggcccggcggctttgattactggggccagggcaccctggtgaccgtctcctct

SEQ ID NO: 32 - DNA, 9109 bp, Artificial Sequence
  pDGB4
tctggctaactagagaacccactgcttactggcttatcgaaattaatacgactcactatagggagacccaagctggctaggccacataggcctgaaccaccatggtgttgcagacccaggtcttcatttctctgttgctctggatctctgtgattacaggtgccgacggggacatcgtgatgacccagtctccagactccctggctgtgtctctgggcgagagggccaccatcaactgcaagtccagccagagtgttttatacagccccaacaatgagaacttcttagcttggtaccaacagaagccaggacagtctcctaagttgctcatttactgggcgtctacccgggaatccggggtccctgaccgattcagtggcagcgggtctgggacagatttcactctcaccatcagcaacctgcaggctgaagatgtggcagtttactactgtcaacaatattatagtgctcctatcactttcggcggagggaccaaggtggagatcaaacgaactgtggctgcaccatctgtcttcatcttcccgccatctgatgagcagttgaaatctggaactgcctctgttgtgtgcctgctgaataacttctatcccagagaggccaaagtacagtggaaggtggataacgccctccaatcgggtaactcccaggagagtgtcacagagcaggacagcaaggacagcacctacagcctcagcagcaccctgacgctgagcaaagcagactacgagaaacacaaactctacgcctgcgaagtcacccatcagggcctgagctcgcccgtcacaaagagcttcaacaggggagagtcttgataaggcctgcacggccctcgagtctagagggcccgtttaaacccgctgatcagcctcgactgtgccttctagttgccagccatctgttgtttgcccctcccccgtgccttccttgaccctggaaggtgccactcccactgtcctttcctaataaaatgaggaaattgcatcgcattgtctgagtaggtgtcattctattctggggggtggggtggggcaggacagcaagggggaggattgggaagacaatagcaggcatgctggggatgcggtgggctctatggcttctgaggcggaaagaaccagctggggctctagggggtatccccacgcgccctgtagcggcgcattaagcgcggcgggtgtggtggttacgcgcagcgtgaccgctacacttgccagcgccctagcgcccgctcctttcgctttcttcccttcctttctcgccacgttcgccggctttccccgtcaagctctaaatcgggggctccctttagggttccgatttagtgctttacggcacctcgaccccaaaaaacttgattagggtgatggttcacgtacctagaagttcctattccgaagttcctattctctagaaagtataggaacttccttggccaaaaagcctgaactcaccgcgacgtctgtcgagaagtttctgatcgaaaagttcgacagcgtgtccgacctgatgcagctctcggagggcgaagaatctcgtgctttcagcttcgatgtaggagggcgtggatatgtcctgcgggtaaatagctgcgccgatggtttctacaaagatcgttatgtttatcggcactttgcatcggccgcgctcccgattccggaagtgcttgacattggggaattcagcgagagcctgacctattgcatctcccgccgtgcacagggtgtcacgttgcaagacctgcctgaaaccgaactgcccgctgttctgcagccggtcgcggaggccatggatgcgatcgctgcggccgatcttagccagacgagcgggttcggcccattcggaccgcaaggaatcggtcaatacactacatggcgtgatttcatatgcgcgattgctgatccccatgtgtatcactggcaaactgtgatggacgacaccgtcagtgcgtccgtcgcgcaggctctcgatgagctgatgctttgggccgaggactgccccgaagtccggcacctcgtgcacgcggatttcggctccaacaatgtcctgacggacaatggccgcataacagcggtcattgactggagcgaggcgatgttcggggattcccaatacgaggtcgccaacatcttcttctggaggccgtggttggcttgtatggagcagcagacgcgctacttcgagcggaggcatccggagcttgcaggatcgccgcggctccgggcgtatatgctccgcattggtcttgaccaactctatcagagcttggttgacggcaatttcgatgatgcagcttgggcgcagggtcgatgcgacgcaatcgtccgatccggagccgggactgtcgggcgtacacaaatcgcccgcagaagcgcggccgtctggaccgatggctgtgtagaagtactcgccgatagtggaaaccgacgccccagcactcgtccgagggcaaaggaatagcacgtactacgagatttcgattccaccgccgccttctatgaaaggttgggcttcggaatcgttttccgggacgccggctggatgatcctccagcgcggggatctcatgctggagttcttcgcccaccccaacttgtttattgcagcttataatggttacaaataaagcaatagcatcacaaatttcacaaataaagcatttttttcactgcattctagttgtggtttgtccaaactcatcaatgtatcttatcatgtctgtataccgtcgacctctagctagagcttggcgtaatcatggtcatagctgtttcctgtgtgaaattgttatccgctcacaattccacacaacatacgagccggaagcataaagtgtaaagcctggggtgcctaatgagtgagctaactcacattaattgcgttgcgctcactgcccgctttccagtcgggaaacctgtcgtgccagctgcattaatgaatcggccaacgcgcggggagaggcggtttgcgtattgggcgctcttccgcttcctcgctcactgactcgctgcgctcggtcgttcggctgcggcgagcggtatcagctcactcaaaggcggtaatacggttatccacagaatcaggggataacgcaggaaagaacatgtgagcaaaaggccagcaaaaggccaggaaccgtaaaaaggccgcgttgctggcgtttttccataggctccgcccccctgacgagcatcacaaaaatcgacgctcaagtcagaggtggcgaaacccgacaggactataaagataccaggcgtttccccctggaagctccctcgtgcgctctcctgttccgaccctgccgcttaccggatacctgtccgcctttctcccttcgggaagcgtggcgctttctcatagctcacgctgtaggtatctcagttcggtgtaggtcgttcgctccaagctgggctgtgtgcacgaaccccccgttcagcccgaccgctgcgccttatccggtaactatcgtcttgagtccaacccggtaagacacgacttatcgccactggcagcagccactggtaacaggattagcagagcgaggtatgtaggcggtgctacagagttcttgaagtggtggcctaactacggctacactagaagaacagtatttggtatctgcgctctgctgaagccagttaccttcggaaaaagagttggtagctcttgatccggcaaacaaaccaccgctggtagcggtggtttttttgtttgcaagcagcagattacgcgcagaaaaaaaggatctcaagaagatcctttgatcttttctacggggtctgacgctcagtggaacgaaaactcacgttaagggattttggtcatgagattatcaaaaaggatcttcacctagatccttttaaattaaaaatgaagttttaaatcaatctaaagtatatatgagtaaacttggtctgacagttaccaatgcttaatcagtgaggcacctatctcagcgatctgtctatttcgttcatccatagttgcctgactccccgtcgtgtagataactacgatacgggagggcttaccatctggccccagtgctgcaatgataccgcgagacccacgctcaccggctccagatttatcagcaataaaccagccagccggaagggccgagcgcagaagtggtcctgcaactttatccgcctccatccagtctattaattgttgccgggaagctagagtaagtagttcgccagttaatagtttgcgcaacgttgttgccattgctacaggcatcgtggtgtcacgctcgtcgtttggtatggcttcattcagctccggttcccaacgatcaaggcgagttacatgatcccccatgttgtgcaaaaaagcggttagctccttcggtcctccgatcgttgtcagaagtaagttggccgcagtgttatcactcatggttatggcagcactgcataattctcttactgtcatgccatccgtaagatgcttttctgtgactggtgagtactcaaccaagtcattctgagaatagtgtatgcggcgaccgagttgctcttgcccggcgtcaatacgggataataccgcgccacatagcagaactttaaaagtgctcatcattggaaaacgttcttcggggcgaaaactctcaaggatcttaccgctgttgagatccagttcgatgtaacccactcgtgcacccaactgatcttcagcatcttttactttcaccagcgtttctgggtgagcaaaaacaggaaggcaaaatgccgcaaaaaagggaataagggcgacacggaaatgttgaatactcatactcttcctttttcaatattattgaagcatttatcagggttattgtctcatgagcggatacatatttgaatgtatttagaaaaataaacaaataggggttccgcgcacatttccccgaaaagtgccacctgacgtcgacggatcgggagatctcccgatcccctatggtgcactctcagtacaatctgctctgatgccgcatagttaagccagtatctgctccctgcttgtgtgttggaggtcgctgagtagtgcgcgagcaaaatttaagctacaacaaggcaaggcttgaccgacaattgcatgaagaatctgcttagggttaggcgttttgcgctgcttcgcgatgtacgggccagatatacgcgttgacattgattattgactagttattaatagtaatcaattacggggtcattagttcatagcccatatatggagttccgcgttacataacttacggtaaatggcccgcctggctgaccgcccaacgacccccgcccattgacgtcaataatgacgtatgttcccatagtaacgccaatagggactttccattgacgtcaatgggtggagtatttacggtaaactgcccacttggcagtacatcaagtgtatcatatgccaagtacgccccctattgacgtcaatgacggtaaatggcccgcctggcattatgcccagtacatgaccttatgggactttcctacttggcagtacatctacgtattagtcatcgctattaccatggtgatgcggttttggcagtacatcaatgggcgtggatagcggtttgactcacggggatttccaagtctccaccccattgacgtcaatgggagtttgttttggcaccaaaatcaacgggactttccaaaatgtcgtaacaactccgccccattgacgcaaatgggcggtaggcgtgtacggtgggaggtctatataagcagagctctctggctaactagagaacccactgcttactggcttatcgaaattaatacgactcactatagggagagggagacccaagctggctagccacctgattggcgtctctagtccaccatggactttgggctgagctggctttttcttgtggctattttaaaaggtgtccagtgtgaggtgcagctgttggagtctgggggaggcttggtacagcctggggggtccctgagactctcctgtgcagcctctggattcacctttagcagctatgccatgagctgggtccgccaggctccagggaaggggctggagtgggtctcaggtattactgggagtggtggtagtacatactacgcagactccgtgaagggccggttcaccatctccagagacaattccaagaacacgctgtatctgcaaatgaacagcctgagagccgaggacacggccgtatattactgtgcgaaagatccagggactacggtgattatgagttggttcgacccctggggccagggaaccctggtcaccgtctcctcagctagcaccaagggcccatcggtcttccccctggcgccctgctccaggagcacctccgagagcacagcggccctgggctgcctggtcaaggactacttccccgaaccggtgacggtgtcgtggaactcaggcgctctgaccagcggcgtgcacaccttcccagctgtcctacagtcctcaggactctactccctcagcagcgtggtgaccgtgccctccagcaacttcggcacccagacctacacctgcaacgtagatcacaagcccagcaacaccaaggtggacaagacagttgagcgcaaatgttgtgtcgagtgcccaccgtgcccagcaccacctgtggcaggaccgtcagtcttcctcttccccccaaaacccaaggacaccctcatgatctcccggacccctgaggtcacgtgcgtggtggtggacgtgagccacgaagaccccgaggtccagttcaactggtacgtggacggcgtggaggtgcataatgccaagacaaagccacgggaggagcagttcaacagcacgttccgtgtggtcagcgtcctcaccgttgtgcaccaggactggctgaacggcaaggagtacaagtgcaaggtctccaacaaaggcctcccagcccccatcgagaaaaccatctccaaaaccaaagggcagccccgagaaccacaggtgtacaccctgcccccatcccgggaggagatgaccaagaaccaggtcagcctgacctgcctggtcaaaggcttctaccccagcgacatcgccgtggagtgggagagcaatgggcagccggagaacaactacaagaccacacctcccatgctggactccgacggctccttcttcctctacagcaagctcaccgtggacaagagcaggtggcagcaggggaacgtcttctcatgctccgtgatgcatgaggctctgcacaaccactacacgcagaagagcctctccctgtctccgggtaaaaatgctgtgggccaggacacgcaggaggtcatcgtggtgccacactccttgccctttaaggtggtggtgatctcagccatcctggccctggtggtgctcaccatcatctcccttatcatcctcatcatgctttggcagaagaagccacgttgataaccatgactctggaccatgggaaatgtcagagtggagaaccacaccgagtgccactgcagcacttgttattatcacaaatcctaatagtttgcagtgggccttgctgatgatggctgacttgctcaaaaggaaaattaatttgtccagtgtctatggctttgtgagataaaaccctccttttccttgccataccatttttaacctgctttgagaatatactgcagctttattgcttttctccttatcctacaatataatcagtagtcttgatcttttcatttggaatgaaatatggcatttagcatgaccataaaaagctgattccactggaaataaagtcttttaaatcatcactctatcactgaattctaattttttctgaaaagtttcaagccagttacttttgataggattaacggaagggagtgagccagtgggtgaggtgggttcccatgtagtcaatggcctaatactggagaatcttattctaaccaagccttccagagcaagctgtgagcccctcagacagtgggctactcatgagacagtccattggggtaaaggaagaaaatataacttctatttctattcatttgcacattgtctttagatgcccatttgggtgagttttatagaagtacagctacattaaaaaatagaactgataatagataaggctttaaaaaaacttcattcatcaccagtttgtcaagattccatttcaaagtgaaaaaccaatttctaacgggttggtaaacacagcagatggcagggtgaaaaattaaagtgagtgcatgtacctttaaagaaacactgaaatgcacacacattacttaacctgctcattcatttatttacatatagtcttgggtgtacaaaatttagaaataaatacatagatctcccgatcccctatggtgcactctcagtacaatctgctctgatgccgcatagttaagccagtatctgctccctgcttgtgtgttggagcaaaatttaagctacaacaaggcaaggcttgaccgacaattgcatgaagaatctgcttagggttaggcgttttgcgctgcttcgcgatgtacgggccagatatacgcgttgacattgattattgactagttattaatagtaatcaattacggggtcattagttcatagcccatatatggagttccgcgttacataacttacggtaaatggcccgcctggctgaccgcccaacgacccccgcccattgacgtcaataatgacgtatgttcccatagtaacgccaatagggactttccattgacgtcaatgggtggagtatttacggtaaactgcccacttggcagtacatcaagtgtatcatatgccaagtacgccccctattgacgtcaatgacggtaaatggcccgcctggcattatgcccagtacatgaccttatgggactttcctacttggcagtacatctacgtattagtcatcgctattaccatggtgatgcggttttggcagtacatcaatgggcgtggatagcggtttgactcacggggatttccaagtctccaccccattgacgtcaatgggagtttgttttggcaccaaaatcaacgggactttccaaaatgtcgtaacaactccgccccattgacgcaaatgggcggtaggcgtgtacggtgggaggtctatataagcagagctc